European Patent Specification EP 4 330 411 B1, published March 18, 2026. Title: Compositions and Methods for Treatment of Ocular Disease Associated with Angiogenesis. Applicant: 4D Molecular Therapeutics, Inc. The sequence listing filed with the application follows.

SEQUENCE LISTING (75 sequences)

SEQ ID NO: 1 - DNA, 21 bp, Artificial Sequence
  Synthetic Polynucleotide
gccgcagcctataacaacttt

SEQ ID NO: 2 - DNA, 21 bp, Artificial Sequence
  Synthetic Polynucleotide
aaagttgttataggctgcggc

SEQ ID NO: 3 - DNA, 21 bp, Artificial Sequence
  Synthetic Polynucleotide
gccgcagcctataacaacttt

SEQ ID NO: 4 - DNA, 21 bp, Artificial Sequence
  Synthetic Polynucleotide
ccctaattctacagaagagat

SEQ ID NO: 5 - DNA, 21 bp, Artificial Sequence
  Synthetic Polynucleotide
atctcttctgtagaattaggg

SEQ ID NO: 6 - DNA, 21 bp, Artificial Sequence
  Synthetic Polynucleotide
ccctaattctacagaagagat

SEQ ID NO: 7 - DNA, 21 bp, Artificial Sequence
  Synthetic Polynucleotide
gatgatagaaatagggacaaa

SEQ ID NO: 8 - DNA, 21 bp, Artificial Sequence
  Synthetic Polynucleotide
tttgtccctatttctatcatc

SEQ ID NO: 9 - DNA, 21 bp, Artificial Sequence
  Synthetic Polynucleotide
gatgatagaaatagggacaaa

SEQ ID NO: 10 - DNA, 21 bp, Artificial Sequence
  Synthetic Polynucleotide
gccacggtgaataattcagtt

SEQ ID NO: 11 - DNA, 21 bp, Artificial Sequence
  Synthetic Polynucleotide
aactgaattattcaccgtggc

SEQ ID NO: 12 - DNA, 21 bp, Artificial Sequence
  Synthetic Polynucleotide
gccacggtgaataattcagtt

SEQ ID NO: 13 - DNA, 21 bp, Artificial Sequence
  Synthetic Polynucleotide
gcttactcattgtatgaacat

SEQ ID NO: 14 - DNA, 21 bp, Artificial Sequence
  Synthetic Polynucleotide
atgttcatacaatgagtaagc

SEQ ID NO: 15 - DNA, 21 bp, Artificial Sequence
  Synthetic Polynucleotide
gcttactcattgtatgaacat

SEQ ID NO: 16 - DNA, 21 bp, Artificial Sequence
  Synthetic Polynucleotide
cgcgacaaacaccttctttaa

SEQ ID NO: 17 - DNA, 21 bp, Artificial Sequence
  Synthetic Polynucleotide
ttaaagaaggtgtttgtcgcg

SEQ ID NO: 18 - DNA, 21 bp, Artificial Sequence
  Synthetic Polynucleotide
cgcgacaaacaccttctttaa

SEQ ID NO: 19 - DNA, 21 bp, Artificial Sequence
  Synthetic Polynucleotide
ctacctcagcaagacgttatt

SEQ ID NO: 20 - DNA, 21 bp, Artificial Sequence
  Synthetic Polynucleotide
aataacgtcttgctgaggtag

SEQ ID NO: 21 - DNA, 21 bp, Artificial Sequence
  Synthetic Polynucleotide
ctacctcagcaagacgttatt

SEQ ID NO: 22 - DNA, 21 bp, Artificial Sequence
  Synthetic Polynucleotide
accaattacatgtggaataat

SEQ ID NO: 23 - DNA, 20 bp, Artificial Sequence
  Synthetic Polynucleotide
attattccacatgtaattgg

SEQ ID NO: 24 - DNA, 21 bp, Artificial Sequence
  Synthetic Polynucleotide
accaattacatgtggaataat

SEQ ID NO: 25 - DNA, 21 bp, Artificial Sequence
  Synthetic Polynucleotide
atgaccaaacagccaagattt

SEQ ID NO: 26 - DNA, 20 bp, Artificial Sequence
  Synthetic Polynucleotide
aaatcttggctgtttggtca

SEQ ID NO: 27 - DNA, 22 bp, Artificial Sequence
  Synthetic Polynucleotide
aatgaccaaacagccaagattt

SEQ ID NO: 28 - DNA, 21 bp, Artificial Sequence
  Synthetic Polynucleotide
gtcgttgtgtcccttcatatt

SEQ ID NO: 29 - DNA, 21 bp, Artificial Sequence
  Synthetic Polynucleotide
aatatgaagggacacaacgac

SEQ ID NO: 30 - DNA, 21 bp, Artificial Sequence
  Synthetic Polynucleotide
gtcgttgtgtcccttcatatt

SEQ ID NO: 31 - DNA, 21 bp, Artificial Sequence
  Synthetic Polynucleotide
acaacggcatccagcgatttc

SEQ ID NO: 32 - DNA, 20 bp, Artificial Sequence
  Synthetic Polynucleotide
gaaatcgctggatgccgttg

SEQ ID NO: 33 - DNA, 21 bp, Artificial Sequence
  Synthetic Polynucleotide
acaacggcatccagcgatttc

SEQ ID NO: 34 - DNA, 21 bp, Artificial Sequence
  Synthetic Polynucleotide
ggacaccctgcaagatgtttg

SEQ ID NO: 35 - DNA, 21 bp, Artificial Sequence
  Synthetic Polynucleotide
caaacatcttgcagggtgtcc

SEQ ID NO: 36 - DNA, 21 bp, Artificial Sequence
  Synthetic Polynucleotide
ggacaccctgcaagatgtttg

SEQ ID NO: 37 - DNA, 21 bp, Artificial Sequence
  Synthetic Polynucleotide
caccgtgtgggctgagtttaa

SEQ ID NO: 38 - DNA, 21 bp, Artificial Sequence
  Synthetic Polynucleotide
ttaaactcagcccacacggtg

SEQ ID NO: 39 - DNA, 21 bp, Artificial Sequence
  Synthetic Polynucleotide
caccgtgtgggctgagtttaa

SEQ ID NO: 40 - DNA, 21 bp, Artificial Sequence
  Synthetic Polynucleotide
ctttaagactttcgctatttc

SEQ ID NO: 41 - DNA, 21 bp, Artificial Sequence
  Synthetic Polynucleotide
gaaatagcgaaagtcttaaag

SEQ ID NO: 42 - DNA, 22 bp, Artificial Sequence
  Synthetic Polynucleotide
ctttaagactttcgctatttcg

SEQ ID NO: 43 - DNA, 21 bp, Artificial Sequence
  Synthetic Polynucleotide
tcacaggcaacgagctctatg

SEQ ID NO: 44 - DNA, 21 bp, Artificial Sequence
  Synthetic Polynucleotide
catagagctcgttgcctgtga

SEQ ID NO: 45 - DNA, 21 bp, Artificial Sequence
  Synthetic Polynucleotide
tcacaggcaacgagctctatg

SEQ ID NO: 46 - RNA, 155 nt, Artificial Sequence
  Synthetic Polynucleotide
  misc_feature (57)..(78): n is a, c, g, u, or absent
  misc_feature (98)..(119): n is a, c, g, u, or absent
cuucagguuaacccaacagaaggcuaaagaagguauauugcuguugacagugagcgnnnnnnnnnnnnnnnnnnnnnncugugaagccacagaugggnnnnnnnnnnnnnnnnnnnnnnugccuacugccucggacuucaaggggcuacuuuagg

SEQ ID NO: 47 - RNA, 153 nt, Artificial Sequence
  Synthetic Polynucleotide
  misc_feature (56)..(77): n is a, c, g, or u
  misc_feature (97)..(118): n is a, c, g, or u
gacuucuuaacccaacagaaggcucgagaagguauauugcuguugacagugagcgnnnnnnnnnnnnnnnnnnnnnnuagugaagccacagauguannnnnnnnnnnnnnnnnnnnnnugccuacugccucggacuucaaggggcuagaauuc

SEQ ID NO: 48 - protein, 745 aa, Artificial Sequence
  Synthetic Polypeptide
MAADGYLPDWLEDTLSEGIRQWWKLKPGPPPPKAAERHKDDSRGLVLPGYKYLGPFNGLDKGEPVNEADAAALEHDKAYDRQLDSGDNPYLKYNHADAEFQERLKEDTSFGGNLGRAVFQAKKRVLEPLGLVEEPVKTAPGKKRPVEHSPVEPDSSSGTGKAGQQPARKRLNFGQTGDADSVPDPQPLGQPPAAPSGLGTNTMATGSGAPMADNNEGADGVGNSSGNWHCDSTWMGDRVITTSTRTWALPTYNNHLYKQISSQSGASNDNHYFGYSTPWGYFDFNRFHCHFSPRDWQRLINNNWGFRPKRLNFKLFNIQVKEVTQNDGTTTIANNLTSTVQVFTDSEYQLPYVLGSAHQGCLPPFPADVFMVPQYGYLTLNNGSQAVGRSSFYCLEYFPSQMLRTGNNFTFSYTFEDVPFHSSYAHSQSLDRLMNPLIDQYLYYLSRTNTPSGTTTQSRLQFSQAGASDIRDQSRNWLPGPCYRQQRVSKTSADNNNSEYSWTGATKYHLNGRDSLVNPGPAMASHKDDEEKFFPQSGVLIFGKQGSEKTNVDIEKVMITDEEEIRTTNPVATEQYGSVSTNLQRGNLAISDQTKHARQAATADVNTQGVLPGMVWQDRDVYLQGPIWAKIPHTDGHFHPSPLMGGFGLKHPPPQILIKNTPVPANPSTTFSAAKFASFITQYSTGQVSVEIEWELQKENSKRWNPEIQYTSNYNKSVNVDFTVDTNGVYSEPRPIGTRYLTRNL

SEQ ID NO: 49 - protein, 10 aa, Artificial Sequence
  Synthetic Polypeptide
LAISDQTKHA

SEQ ID NO: 50 - DNA, 1374 bp, Artificial Sequence
  Synthetic Polynucleotide
atggtttcttactgggacaccggcgtgctgctgtgtgccctgctttcttgtctgctgctgaccggctctagcagcggctctgataccggcagacccttcgtggaaatgtacagcgagatccccgagatcatccacatgaccgagggcagagagctggtcatcccttgcagagtgacaagccccaacatcaccgtgactctgaagaagttccctctggacacactgatccccgacggcaagagaatcatctgggacagccggaagggcttcatcatcagcaacgccacctacaaagagatcggcctgctgacctgtgaagccaccgtgaatggccacctgtacaagaccaactacctgacacacagacagaccaacaccatcatcgacgtggtgctgagccctagccacggcattgaactgtctgtgggcgagaagctggtgctgaactgtaccgccagaaccgagctgaacgtgggcatcgacttcaactgggagtaccccagcagcaagcaccagcacaagaaactggtcaaccgggacctgaaaacccagagcggcagcgagatgaagaaattcctgagcaccctgaccatcgacggcgtgaccagaagtgaccagggcctgtacacatgtgccgccagctctggcctgatgaccaagaaaaacagcaccttcgtgcgggtgcacgagaaggacaagacccacacctgtcctccatgtcctgctccagaactgctcggcggaccttccgtgttcctgtttcctccaaagcctaaggacaccctgatgatcagcagaacccctgaagtgacctgcgtggtggtggatgtgtcccacgaggatcccgaagtgaagttcaattggtacgtggacggcgtggaagtgcacaacgccaagaccaagcctagagaggaacagtacaatagcacctacagagtggtgtccgtgctgaccgtgctgcaccaggattggctgaacggcaaagagtacaagtgcaaggtgtccaacaaggccctgcctgctcctatcgagaaaaccatctccaaggccaagggccagcctagggaaccccaggtttacacactgcctccaagcagggacgagctgacaaagaaccaggtgtccctgacctgcctggtcaagggcttctacccttccgatatcgccgtggaatgggagagcaatggccagcctgagaacaactacaagacaacccctcctgtgctggacagcgacggctcattcttcctgtacagcaagctgacagtggacaagagcagatggcagcagggcaacgtgttcagctgctccgtgatgcacgaggccctgcacaaccactacacccagaagtccctgagcctgtctcctggcaaa

SEQ ID NO: 51 - protein, 458 aa, Artificial Sequence
  Synthetic Polypeptide
MVSYWDTGVLLCALLSCLLLTGSSSGSDTGRPFVEMYSEIPEIIHMTEGRELVIPCRVTSPNITVTLKKFPLDTLIPDGKRIIWDSRKGFIISNATYKEIGLLTCEATVNGHLYKTNYLTHRQTNTIIDVVLSPSHGIELSVGEKLVLNCTARTELNVGIDFNWEYPSSKHQHKKLVNRDLKTQSGSEMKKFLSTLTIDGVTRSDQGLYTCAASSGLMTKKNSTFVRVHEKDKTHTCPPCPAPELLGGPSVFLFPPKPKDTLMISRTPEVTCVVVDVSHEDPEVKFNWYVDGVEVHNAKTKPREEQYNSTYRVVSVLTVLHQDWLNGKEYKCKVSNKALPAPIEKTISKAKGQPREPQVYTLPPSRDELTKNQVSLTCLVKGFYPSDIAVEWESNGQPENNYKTTPPVLDSDGSFFLYSKLTVDKSRWQQGNVFSCSVMHEALHNHYTQKSLSLSPGK

SEQ ID NO: 52 - protein, 5 aa, Artificial Sequence
  Synthetic Polypeptide
GYYMH

SEQ ID NO: 53 - protein, 17 aa, Artificial Sequence
  Synthetic Polypeptide
WINPNSGGTNYAQKFQG

SEQ ID NO: 54 - protein, 20 aa, Artificial Sequence
  Synthetic Polypeptide
SPNPYYYDSSGYYYPGAFDI

SEQ ID NO: 55 - protein, 11 aa, Artificial Sequence
  Synthetic Polypeptide
GGNNIGSKSVH

SEQ ID NO: 56 - protein, 7 aa, Artificial Sequence
  Synthetic Polypeptide
DDSDRPS

SEQ ID NO: 57 - protein, 11 aa, Artificial Sequence
  Synthetic Polypeptide
QVWDSSSDHWV

SEQ ID NO: 58 - DNA, 1686 bp, Artificial Sequence
  Synthetic Polynucleotide
atgcaaagaggcgccgctctctgtctgagactgtggctgtgtctgggcctgctggatggactggtgtctggctacagcatgacccctccaacactgaacatcaccgaggaatcccacgtgatcgacaccggcgatagcctgagcatcagctgcagaggacagcaccctctggaatgggcttggcctggtgctcaagaagctcctgccacaggcgacaaggacagcgaggatacaggcgttgtgcgggattgcgagggcacagatgccagaccttactgcaaggtgctgctgctgcacgaagtgcacgcccaggataccggcagctacgtgtgctactacaagtacatcaaggcccggatcgagggcaccacagccgcaagctcttatgtgttcgtgcgggacttcgagcagcccttcatcaacaagcccgacacactgctggtcaaccggaaggacgctatgtgggtgccctgtctggtgtctatccccggcctgaatgtgaccctgagaagccagagttccgtgctgtggcctgatggccaagaggtcgtgtgggacgatagaaggggcatgctggtgtccacacctctgctgcatgatgccctgtacctgcagtgcgagacaacctggggcgaccaggacttcctgagcaaccctttcctggtgcacatcaccggcaacgagctgtacgacatccagctgctgcctcgcaagagcctggaactgctcgtgggagagaagctggtgctgaactgtaccgtgtgggccgagttcaatagcggcgtgaccttcgactgggactaccctggaaagcaggccgagcgtggaaaatgggtgcccgagagaagaagccagcagacccacacagagctgagcagcatcctgaccatccacaacgtgtcccagcacgatctgggctcttacgtgtgcaaggccaacaacggcatccagcggttccgggaaagcaccgaagtgatcgtgcatgaggaacccaagagctgcgacaagacacacacctgtcctccatgtcctgctccagagcttctcggcggaccttccgtgttcctgtttcctccaaagcctaaggacaccctgatgatcagcagaacccctgaagtgacctgcgtggtggtggatgtgtcccacgaggatcccgaagtgaagttcaattggtacgtggacggcgtggaagtgcacaatgccaagaccaagcctagagaggaacagtacaacagcacctacagagtggtgtccgtgctgaccgtgctgcatcaggattggctgaacggcaaagagtacaagtgcaaggtgtccaacaaggccctgcctgctcctatcgagaaaaccatctccaaggccaagggccagcctcgggaacctcaagtgtataccctgcctcctagccgcgacgaactcaccaagaatcaagtgtctctgacatgtctcgtgaaggggttttaccccagcgacattgccgtcgagtgggagtccaatggacaacccgagaacaattataagaccacgccaccagtcctggactccgacggctcattttttctctactccaaactgaccgtggataagtcccggtggcagcaagggaatgtgttttcctgtagcgtgatgcatgaagctctccacaatcattacacccaaaaatctctgtctctgagccccggcaaatga

SEQ ID NO: 59 - protein, 1674 aa, Artificial Sequence
  Synthetic Polypeptide
ATGCAGAGGGGAGCCGCCCTGTGCCTGAGGCTGTGGCTGTGCCTGGGCCTGCTGGACGGCCTGGTGTCTGGCTACAGCATGACCCCCCCTACACTGAACATCACCGAGGAGAGCCACGTGATCGACACAGGCGATAGCCTGTCCATCTCTTGCAGGGGCCAGCACCCCCTGGAGTGGGCATGGCCTGGAGCACAGGAGGCACCAGCCACCGGCGACAAGGATAGCGAGGACACAGGAGTGGTGCGGGACTGCGAGGGAACCGATGCCAGACCTTACTGTAAGGTGCTGCTGCTGCACGAGGTGCACGCCCAGGATACAGGCTCCTACGTGTGCTACTATAAGTATATCAAGGCAAGGATCGAGGGAACCACAGCAGCCAGCTCCTACGTGTTCGTGCGGGATTTTGAGCAGCCTTTCATCAACAAGCCAGACACCCTGCTGGTGAATCGGAAGGATGCCATGTGGGTGCCCTGTCTGGTGTCTATCCCTGGCCTGAATGTGACACTGAGAAGCCAGTCTAGCGTGCTGTGGCCAGACGGACAGGAGGTGGTGTGGGACGATCGGAGAGGCATGCTGGTGAGCACCCCTCTGCTGCACGATGCCCTGTACCTGCAGTGCGAGACAACATGGGGCGACCAGGATTTTCTGTCCAACCCTTTCCTGGTGCACATCACAGGCAATGAGCTGTATGACATCCAGCTGCTGCCACGGAAGTCCCTGGAGCTGCTGGTGGGCGAGAAGCTGGTGCTGAACTGTACCGTGTGGGCCGAGTTTAATTCTGGCGTGACATTCGACTGGGATTACCCCGGCAAGCAGGCCGAGAGGGGCAAGTGGGTGCCTGAGAGGCGCAGCCAGCAGACCCACACAGAGCTGTCCTCTATCCTGACCATCCACAACGTGAGCCAGCACGATCTGGGCTCCTACGTGTGCAAGGCCAACAATGGCATCCAGCGGTTTAGAGAGTCTACAGAAGTGATCGTGCACGAGGAGAGGAAGTGCTGCGTGGAGTGCCCACCATGTCCAGCACCTCCAGTGGCAGGACCATCCGTGTTCCTGTTTCCACCTAAGCCTAAGGACACCCTGATGATCAGCCGCACCCCAGAGGTGACATGCGTGGTGGTGGACGTGTCCCACGAGGATCCAGAGGTGCAGTTCAACTGGTACGTGGATGGCGTGGAGGTGCACAATGCCAAGACCAAGCCCAGGGAGGAGCAGTTTAATTCTACCTTCCGCGTGGTGAGCGTGCTGACAGTGGTGCACCAGGACTGGCTGAACGGCAAGGAGTATAAGTGCAAGGTGTCTAATAAGGGCCTGCCCGCCCCTATCGAGAAGACCATCAGCAAGACAAAGGGACAGCCACGGGAGCCACAGGTGTACACCCTGCCACCATCCAGAGAGGAGATGACCAAGAACCAGGTGTCTCTGACATGTCTGGTGAAGGGCTTTTATCCAAGCGACATCGCCGTGGAGTGGGAGTCCAATGGCCAGCCCGAGAACAATTACAAGACCACACCTCCAATGCTGGACTCCGATGGCTCTTTCTTTCTGTATTCCAAGCTGACCGTGGATAAGTCTCGGTGGCAGCAGGGCAACGTGTTCAGCTGTTCCGTGATGCACGAGGCCCTGCACAATCACTACACACAGAAGTCTCTGAGCCTGTCCCCCGGCAAGTGA

SEQ ID NO: 60 - DNA, 1257 bp, Artificial Sequence
  Synthetic Polynucleotide
atgcaagctctggtgctgctgctgtgtatcggagccctgctgggccacagctcctgtcaaaatcctgcctctccacctgaggaaggcagccccgatccagattctacaggcgccctggtggaagaagaggacccattcttcaaggtgcccgtgaacaaactggccgctgccgtgtccaacttcggctacgacctgtacagagtgcggagcagcacaagccccaccaccaatgttctgctgagccctctgtctgtggccaccgctctttctgctctgtctctgggagccgagcagagaaccgagagcatcattcacagagccctgtactacgatctgatcagcagccctgacatccacggcacctacaaagaactgctggacaccgtgacagcccctcagaagaatctgaagtccgccagccggatcgtgttcgagaagaagctgcggatcaagagcagcttcgtggcccctctggaaaagagctacggcaccagacctagagtgctgaccggcaatcccagactggacctgcaagagatcaacaactgggtgcaagcccagatgaagggcaagctggccagaagcaccaaagagatccccgacgagatcagcatcctgctgctgggcgtcgcccactttaaaggccagtgggtcaccaagttcgactccagaaagaccagcctcgaggacttctacctggacgaggaacggaccgtcagagtgcccatgatgagcgatcctaaggccgtgctgagatacggcctggatagcgacctgagctgcaagattgctcagctgcctctgaccggctctatgagcatcatattctttctgcccctgaaagtgacccagaatctgaccctgatcgaggaaagcctgaccagcgagttcatccacgacatcgaccgcgagctgaaaaccgtgcaggctgtgctgactgtgcccaagctgaagctgagctacgagggcgaagtgaccaagagcctgcaagaaatgaagctgcagagcctgttcgacagccccgacttcagcaagatcaccggcaagcccatcaagctgacccaggtggaacacagagccggcttcgagtggaatgaagatggcgccggaaccacaccttctccaggactgcaacctgctcacctgacctttccactggactaccacctgaaccagcctttcatcttcgtgctgcgggacacagatactggcgccctgctgttcatcggcaagatcctggatcctagaggcccctga

SEQ ID NO: 61 - DNA, 145 bp, adeno-associated virus 2
ttggccactccctctctgcgcgctcgctcgctcactgaggccgggcgaccaaaggtcgcccgacgcccgggctttgcccgggcggcctcagtgagcgagcgagcgcgcagagagggagtggccaactccatcactaggggttcct

SEQ ID NO: 62 - DNA, 145 bp, adeno-associated virus 2
aggaacccctagtgatggagttggccactccctctctgcgcgctcgctcgctcactgaggccgcccgggcaaagcccgggcgtcgggcgacctttggtcgcccggcctcagtgagcgagcgagcgcgcagagagggagtggccaa

SEQ ID NO: 63 - DNA, 245 bp, Artificial Sequence
  Synthetic Polynucleotide
ggggatccagacatgataagatacattgatgagtttggacaaaccacaactagaatgcagtgaaaaaaatgctttatttgtgaaatttgtgatgctattgctttatttgtaaccattataagctgcaataaacaagttaacaacaacaattgcattcattttatgtttcaggttcagggggaggtgtgggaggttttttaaagcaagtaaaacctctacaaatgtggtatggctgattatgatca

SEQ ID NO: 64 - DNA, 4297 bp, Artificial Sequence
  Synthetic Polynucleotide
ttggccactccctctctgcgcgctcgctcgctcactgaggccgggcgaccaaaggtcgcccgacgcccgggctttgcccgggcggcctcagtgagcgagcgagcgcgcagagagggagtggccaactccatcactaggggttcctatcgattgaattccaggcgcgccatcctgcaggtattgacgtcaataatgacgtatgttcccatagtaacgccaatagggactttccattgacgtcaatgggtggagtatttacggtaaactgcccacttggcagtacatcaagtgtatcatatgccaagtacgccccctattgacgtcaatgacggtaaatggcccgcctggcattatgcccagtacatgaccttatgggactttcctacttggcagtacatctacgtattagtcatcgctattaccatggtcgaggtgagccccacgttctgcttcactctccccatctcccccccctccccacccccaattttgtatttatttattttttaattattttgtgcagcgatgggggcggggggggggggggggcgcgcgccaggcggggcggggcggggcgaggggcggggcggggcgaggcggagaggtgcggcggcagccaatcagagcggcgcgctccgaaagtttccttttatggcgaggcggcggcggcggcggccctataaaaagcgaagcgcgcggcgggcgggagtcgctgcgcgctgccttcgccccgtgccccgctccgccgccgcctcgcgccgcccgccccggctctgactgaccgcgttactcccacaggtgagcgggcgggacggcccttctcctccgggctgtaattagcgcttggtttaatgacggcttgtttcttttctgtggctgcgtgaaagccttgaggggctccgggagggccctttgtgcggggggagcggctcggggctgtccgcggggggacggctgccttcgggggggacggggcagggcggggttcggcttctggcgtgtgaccggcggctctagagcctctgctaaccatgttcatgccttcttctttttcctacagctcctgggcaacgtgctggttattgtgctgtctcatcattttggcaaagaattgtacaggatatcttgctagcacgccaccatggtttcttactgggacaccggcgtgctgctgtgtgccctgctttcttgtctgctgctgaccggctctagcagcggctctgataccggcagacccttcgtggaaatgtacagcgagatccccgagatcatccacatgaccgagggcagagagctggtcatcccttgcagagtgacaagccccaacatcaccgtgactctgaagaagttccctctggacacactgatccccgacggcaagagaatcatctgggacagccggaagggcttcatcatcagcaacgccacctacaaagagatcggcctgctgacctgtgaagccaccgtgaatggccacctgtacaagaccaactacctgacacacagacagaccaacaccatcatcgacgtggtgctgagccctagccacggcattgaactgtctgtgggcgagaagctggtgctgaactgtaccgccagaaccgagctgaacgtgggcatcgacttcaactgggagtaccccagcagcaagcaccagcacaagaaactggtcaaccgggacctgaaaacccagagcggcagcgagatgaagaaattcctgagcaccctgaccatcgacggcgtgaccagaagtgaccagggcctgtacacatgtgccgccagctctggcctgatgaccaagaaaaacagcaccttcgtgcgggtgcacgagaaggacaagacccacacctgtcctccatgtcctgctccagaactgctcggcggaccttccgtgttcctgtttcctccaaagcctaaggacaccctgatgatcagcagaacccctgaagtgacctgcgtggtggtggatgtgtcccacgaggatcccgaagtgaagttcaattggtacgtggacggcgtggaagtgcacaacgccaagaccaagcctagagaggaacagtacaatagcacctacagagtggtgtccgtgctgaccgtgctgcaccaggattggctgaacggcaaagagtacaagtgcaaggtgtccaacaaggccctgcctgctcctatcgagaaaaccatctccaaggccaagggccagcctagggaaccccaggtttacacactgcctccaagcagggacgagctgacaaagaaccaggtgtccctgacctgcctggtcaagggcttctacccttccgatatcgccgtggaatgggagagcaatggccagcctgagaacaactacaagacaacccctcctgtgctggacagcgacggctcattcttcctgtacagcaagctgacagtggacaagagcagatggcagcagggcaacgtgttcagctgctccgtgatgcacgaggccctgcacaaccactacacccagaagtccctgagcctgtctcctggcaaacggaagagaagaggcagcggcgaaggcagaggatccctgcttacatgtggcgacgtggaagagaaccccggacctatgcaagctctggtgctgctgctgtgtatcggagccctgctgggccacagctcctgtcaaaatcctgcctctccacctgaggaaggcagccccgatccagattctacaggcgccctggtggaagaagaggacccattcttcaaggtgcccgtgaacaaactggccgctgccgtgtccaacttcggctacgacctgtacagagtgcggagcagcacaagccccaccaccaatgttctgctgagccctctgtctgtggccaccgctctttctgctctgtctctgggagccgagcagagaaccgagagcatcattcacagagccctgtactacgatctgatcagcagccctgacatccacggcacctacaaagaactgctggacaccgtgacagcccctcagaagaatctgaagtccgccagccggatcgtgttcgagaagaagctgcggatcaagagcagcttcgtggcccctctggaaaagagctacggcaccagacctagagtgctgaccggcaatcccagactggacctgcaagagatcaacaactgggtgcaagcccagatgaagggcaagctggccagaagcaccaaagagatccccgacgagatcagcatcctgctgctgggcgtcgcccactttaaaggccagtgggtcaccaagttcgactccagaaagaccagcctcgaggacttctacctggacgaggaacggaccgtcagagtgcccatgatgagcgatcctaaggccgtgctgagatacggcctggatagcgacctgagctgcaagattgctcagctgcctctgaccggctctatgagcatcatattctttctgcccctgaaagtgacccagaatctgaccctgatcgaggaaagcctgaccagcgagttcatccacgacatcgaccgcgagctgaaaaccgtgcaggctgtgctgactgtgcccaagctgaagctgagctacgagggcgaagtgaccaagagcctgcaagaaatgaagctgcagagcctgttcgacagccccgacttcagcaagatcaccggcaagcccatcaagctgacccaggtggaacacagagccggcttcgagtggaatgaagatggcgccggaaccacaccttctccaggactgcaacctgctcacctgacctttccactggactaccacctgaaccagcctttcatcttcgtgctgcgggacacagatactggcgccctgctgttcatcggcaagatcctggatcctagaggcccctgagccacgcgtaacacgtgcatgcgagagatctgcggccgcgagctcggggatccagacatgataagatacattgatgagtttggacaaaccacaactagaatgcagtgaaaaaaatgctttatttgtgaaatttgtgatgctattgctttatttgtaaccattataagctgcaataaacaagttaacaacaacaattgcattcattttatgtttcaggttcagggggaggtgtgggaggttttttaaagcaagtaaaacctctacaaatgtggtatggctgattatgatcaatgcatcctagccggaggaacccctagtgatggagttggccactccctctctgcgcgctcgctcgctcactgaggccgcccgggcaaagcccgggcgtcgggcgacctttggtcgcccggcctcagtgagcgagcgagcgcgcagagagggagtggccaa

SEQ ID NO: 65 - DNA, 4726 bp, Artificial Sequence
  Synthetic Polynucleotide
ttggccactccctctctgcgcgctcgctcgctcactgaggccgggcgaccaaaggtcgcccgacgcccgggctttgcccgggcggcctcagtgagcgagcgagcgcgcagagagggagtggccaactccatcactaggggttcctatcgattgaattccaggcgcgccatcctgcaggtattgacgtcaataatgacgtatgttcccatagtaacgccaatagggactttccattgacgtcaatgggtggagtatttacggtaaactgcccacttggcagtacatcaagtgtatcatatgccaagtacgccccctattgacgtcaatgacggtaaatggcccgcctggcattatgcccagtacatgaccttatgggactttcctacttggcagtacatctacgtattagtcatcgctattaccatggtcgaggtgagccccacgttctgcttcactctccccatctcccccccctccccacccccaattttgtatttatttattttttaattattttgtgcagcgatgggggcggggggggggggggggcgcgcgccaggcggggcggggcggggcgaggggcggggcggggcgaggcggagaggtgcggcggcagccaatcagagcggcgcgctccgaaagtttccttttatggcgaggcggcggcggcggcggccctataaaaagcgaagcgcgcggcgggcgggagtcgctgcgcgctgccttcgccccgtgccccgctccgccgccgcctcgcgccgcccgccccggctctgactgaccgcgttactcccacaggtgagcgggcgggacggcccttctcctccgggctgtaattagcgcttggtttaatgacggcttgtttcttttctgtggctgcgtgaaagccttgaggggctccgggagggccctttgtgcggggggagcggctcggggctgtccgcggggggacggctgccttcgggggggacggggcagggcggggttcggcttctggcgtgtgaccggcggctctagagcctctgctaaccatgttcatgccttcttctttttcctacagctcctgggcaacgtgctggttattgtgctgtctcatcattttggcaaagaattgtacaggatatcttgctagcacgccaccatggtttcttactgggacaccggcgtgctgctgtgtgccctgctttcttgtctgctgctgaccggctctagcagcggctctgataccggcagacccttcgtggaaatgtacagcgagatccccgagatcatccacatgaccgagggcagagagctggtcatcccttgcagagtgacaagccccaacatcaccgtgactctgaagaagttccctctggacacactgatccccgacggcaagagaatcatctgggacagccggaagggcttcatcatcagcaacgccacctacaaagagatcggcctgctgacctgtgaagccaccgtgaatggccacctgtacaagaccaactacctgacacacagacagaccaacaccatcatcgacgtggtgctgagccctagccacggcattgaactgtctgtgggcgagaagctggtgctgaactgtaccgccagaaccgagctgaacgtgggcatcgacttcaactgggagtaccccagcagcaagcaccagcacaagaaactggtcaaccgggacctgaaaacccagagcggcagcgagatgaagaaattcctgagcaccctgaccatcgacggcgtgaccagaagtgaccagggcctgtacacatgtgccgccagctctggcctgatgaccaagaaaaacagcaccttcgtgcgggtgcacgagaaggacaagacccacacctgtcctccatgtcctgctccagaactgctcggcggaccttccgtgttcctgtttcctccaaagcctaaggacaccctgatgatcagcagaacccctgaagtgacctgcgtggtggtggatgtgtcccacgaggatcccgaagtgaagttcaattggtacgtggacggcgtggaagtgcacaacgccaagaccaagcctagagaggaacagtacaatagcacctacagagtggtgtccgtgctgaccgtgctgcaccaggattggctgaacggcaaagagtacaagtgcaaggtgtccaacaaggccctgcctgctcctatcgagaaaaccatctccaaggccaagggccagcctagggaaccccaggtttacacactgcctccaagcagggacgagctgacaaagaaccaggtgtccctgacctgcctggtcaagggcttctacccttccgatatcgccgtggaatgggagagcaatggccagcctgagaacaactacaagacaacccctcctgtgctggacagcgacggctcattcttcctgtacagcaagctgacagtggacaagagcagatggcagcagggcaacgtgttcagctgctccgtgatgcacgaggccctgcacaaccactacacccagaagtccctgagcctgtctcctggcaaacggaagagaagaggcagcggcgaaggcagaggatccctgcttacatgtggcgacgtggaagagaaccccggacctatgcaaagaggcgccgctctctgtctgagactgtggctgtgtctgggcctgctggatggactggtgtctggctacagcatgacccctccaacactgaacatcaccgaggaatcccacgtgatcgacaccggcgatagcctgagcatcagctgcagaggacagcaccctctggaatgggcttggcctggtgctcaagaagctcctgccacaggcgacaaggacagcgaggatacaggcgttgtgcgggattgcgagggcacagatgccagaccttactgcaaggtgctgctgctgcacgaagtgcacgcccaggataccggcagctacgtgtgctactacaagtacatcaaggcccggatcgagggcaccacagccgctagctcttatgtgttcgtgcgggacttcgagcagcccttcatcaacaagcccgacacactgctggtcaaccggaaggacgctatgtgggtgccctgtctggtgtctatccccggcctgaatgtgaccctgagaagccagagttccgtgctgtggcctgatggccaagaggtcgtgtgggacgatagaaggggcatgctggtgtccacacctctgctgcatgatgccctgtacctgcagtgcgagacaacctggggcgaccaggacttcctgagcaaccctttcctggtgcacatcaccggcaacgagctgtacgacatccagctgctgcctcgcaagagcctggaactgctcgtgggagagaagctggtgctgaactgtaccgtgtgggccgagttcaatagcggcgtgaccttcgactgggactaccctggaaagcaggccgagcgtggaaaatgggtgcccgagagaagaagccagcagacccacacagagctgagcagcatcctgaccatccacaacgtgtcccagcacgatctgggctcttacgtgtgcaaggccaacaacggcatccagcggttccgggaaagcaccgaagtgatcgtgcatgaggaacccaagagctgcgacaagacacacacctgtcctccatgtcctgctccagagcttctcggcggaccttccgtgttcctgtttcctccaaagcctaaggacaccctgatgatcagcagaacccctgaagtgacctgcgtggtggtggatgtgtcccacgaggatcccgaagtgaagttcaattggtacgtggacggcgtggaagtgcacaatgccaagaccaagcctagagaggaacagtacaacagcacctacagagtggtgtccgtgctgaccgtgctgcatcaggattggctgaacggcaaagagtacaagtgcaaggtgtccaacaaggccctgcctgctcctatcgagaaaaccatctccaaggccaagggccagcctcgggaacctcaagtgtataccctgcctcctagccgcgacgaactcaccaagaatcaagtgtctctgacatgtctcgtgaaggggttttaccccagcgacattgccgtcgagtgggagtccaatggacaacccgagaacaattataagaccacgccaccagtcctggactccgacggctcattttttctctactccaaactgaccgtggataagtcccggtggcagcaagggaatgtgttttcctgtagcgtgatgcatgaagctctccacaatcattacacccaaaaatctctgtctctgagccccggcaaatgagccacgcgtaacacgtgcatgcgagagatctgcggccgcgagctcggggatccagacatgataagatacattgatgagtttggacaaaccacaactagaatgcagtgaaaaaaatgctttatttgtgaaatttgtgatgctattgctttatttgtaaccattataagctgcaataaacaagttaacaacaacaattgcattcattttatgtttcaggttcagggggaggtgtgggaggttttttaaagcaagtaaaacctctacaaatgtggtatggctgattatgatcaatgcatcctagccggaggaacccctagtgatggagttggccactccctctctgcgcgctcgctcgctcactgaggccgcccgggcaaagcccgggcgtcgggcgacctttggtcgcccggcctcagtgagcgagcgagcgcgcagagagggagtggccaa

SEQ ID NO: 66 - DNA, 4642 bp, Artificial Sequence
  Synthetic Polynucleotide
ttggccactccctctctgcgcgctcgctcgctcactgaggccgggcgaccaaaggtcgcccgacgcccgggctttgcccgggcggcctcagtgagcgagcgagcgcgcagagagggagtggccaactccatcactaggggttcctatcgattgaattccaggcgcgccatcctgcaggtattgacgtcaataatgacgtatgttcccatagtaacgccaatagggactttccattgacgtcaatgggtggagtatttacggtaaactgcccacttggcagtacatcaagtgtatcatatgccaagtacgccccctattgacgtcaatgacggtaaatggcccgcctggcattatgcccagtacatgaccttatgggactttcctacttggcagtacatctacgtattagtcatcgctattaccatggtcgaggtgagccccacgttctgcttcactctccccatctcccccccctccccacccccaattttgtatttatttattttttaattattttgtgcagcgatgggggcggggggggggggggggcgcgcgccaggcggggcggggcggggcgaggggcggggcggggcgaggcggagaggtgcggcggcagccaatcagagcggcgcgctccgaaagtttccttttatggcgaggcggcggcggcggcggccctataaaaagcgaagcgcgcggcgggcgggagtcgctgcgcgctgccttcgccccgtgccccgctccgccgccgcctcgcgccgcccgccccggctctgactgaccgcgttactcccacaggtgagcgggcgggacggcccttctcctccgggctgtaattagcgcttggtttaatgacggcttgtttcttttctgtggctgcgtgaaagccttgaggggctccgggagggccctttgtgcggggggagcggctcggggctgtccgcggggggacggctgccttcgggggggacggggcagggcggggttcggcttctggcgtgtgaccggcggctctagagcctctgctaaccatgttcatgccttcttctttttcctacagctcctgggcaacgtgctggttattgtgctgtctcatcattttggcaaagaattgtacaggatatcttgctagcacgccaccatggtttcttactgggacaccggcgtgctgctgtgtgccctgctttcttgtctgctgctgaccggctctagcagcggctctgataccggcagacccttcgtggaaatgtacagcgagatccccgagatcatccacatgaccgagggcagagagctggtcatcccttgcagagtgacaagccccaacatcaccgtgactctgaagaagttccctctggacacactgatccccgacggcaagagaatcatctgggacagccggaagggcttcatcatcagcaacgccacctacaaagagatcggcctgctgacctgtgaagccaccgtgaatggccacctgtacaagaccaactacctgacacacagacagaccaacaccatcatcgacgtggtgctgagccctagccacggcattgaactgtctgtgggcgagaagctggtgctgaactgtaccgccagaaccgagctgaacgtgggcatcgacttcaactgggagtaccccagcagcaagcaccagcacaagaaactggtcaaccgggacctgaaaacccagagcggcagcgagatgaagaaattcctgagcaccctgaccatcgacggcgtgaccagaagtgaccagggcctgtacacatgtgccgccagctctggcctgatgaccaagaaaaacagcaccttcgtgcgggtgcacgagaaggacaagacccacacctgtcctccatgtcctgctccagaactgctcggcggaccttccgtgttcctgtttcctccaaagcctaaggacaccctgatgatcagcagaacccctgaagtgacctgcgtggtggtggatgtgtcccacgaggatcccgaagtgaagttcaattggtacgtggacggcgtggaagtgcacaacgccaagaccaagcctagagaggaacagtacaatagcacctacagagtggtgtccgtgctgaccgtgctgcaccaggattggctgaacggcaaagagtacaagtgcaaggtgtccaacaaggccctgcctgctcctatcgagaaaaccatctccaaggccaagggccagcctagggaaccccaggtttacacactgcctccaagcagggacgagctgacaaagaaccaggtgtccctgacctgcctggtcaagggcttctacccttccgatatcgccgtggaatgggagagcaatggccagcctgagaacaactacaagacaacccctcctgtgctggacagcgacggctcattcttcctgtacagcaagctgacagtggacaagagcagatggcagcagggcaacgtgttcagctgctccgtgatgcacgaggccctgcacaaccactacacccagaagtccctgagcctgtctcctggcaaacggaagagaagaggcagcggcgaaggcagaggatccctgcttacatgtggcgacgtggaagagaaccccggacctatggattggacctggtccatcctgtttctggtggccgctgccacaggcacatactctcaggttcagctggtgcagtctggcgccgaagtgaaaaaacctggcgcctccgtgaaggtgtcctgcaaggctagcggctacacctttaccggctactacatgcactgggtccgacaggctccaggacagggacttgaatggatgggctggatcaaccccaatagcggcggcaccaattacgcccagaaattccagggcagagtgaccatgaccagagacaccagcatcagcaccgcctacatggaactgagccggctgagatccgatgacaccgccgtgtactactgcgccagatctcccaatccttactactacgacagcagcgggtactactacccaggcgcctttgatatctggggccagggcacaatggtcaccgtgtcatctgcatctgtggccgctcctagcgtgttcatcttcccaccttccgacgaacagctgaagtctggcacagccagcgtcgtgtgcctgctgaacaacttctaccccagagaagccaaggtgcagtggaaggtggacaacgctctgcagtccggcaacagccaagagagcgtgacagagcaggacagcaaggactccacctacagcctgagcagcaccctgacactgagcaaggccgactacgagaagcacaaagtgtacgcctgcgaagtgacccaccagggcctttctagccctgtgaccaagagcttcaaccggggcgagtgcgataagacacacacaggcggaagcagcggcagcggatctggatctaccggcacatctagctctggcaccggaacatctgccggcacaactggcacaagcgcctctacatctggaagcggttctggcggaggcggaggatctggtggtggtggatctgctggcggaacagctacagctggcgcttctagcggcagcagctatgtgctgacacagcctccatccgtgtctgtggcacctggacagaccgccagaattacctgtggcggcaacaacatcggcagcaagagcgtgcactggtatcagcagaagcctggacaggcaccagtgctggtggtgtacgacgacagcgatagacctagcggcatccccgagagattcagcggctctaacagcggcaataccgccacactgaccatcagcagagtggaagctggcgacgaggccgattactactgccaagtgtgggacagcagcagcgaccactgggttttcggcggaggcaccaaactgacagtgctgtctagcgccagcacaaagggcccatctgtgttccctctggctcccagcagcaagtctacaagcggaggaacagccgctctgggctgcctcgtgaaggattactttcccgagcctgtgaccgtgtcctggaatagcggagcactgacaagcggcgtgcacacctttccagctgtgctgcaaagctccggcctgtactctctgagcagcgtggtcacagtgcctagctctagcctgggcacccagacctacatctgcaatgtgaaccacaagcctagcaacaccaaggtcgacaagaaggtggaacccaagagctgctgagccacgcgtaacacgtgcatgcgagagatctgcggccgcgagctcggggatccagacatgataagatacattgatgagtttggacaaaccacaactagaatgcagtgaaaaaaatgctttatttgtgaaatttgtgatgctattgctttatttgtaaccattataagctgcaataaacaagttaacaacaacaattgcattcattttatgtttcaggttcagggggaggtgtgggaggttttttaaagcaagtaaaacctctacaaatgtggtatggctgattatgatcaatgcatcctagccggaggaacccctagtgatggagttggccactccctctctgcgcgctcgctcgctcactgaggccgcccgggcaaagcccgggcgtcgggcgacctttggtcgcccggcctcagtgagcgagcgagcgcgcagagagggagtggccaa

SEQ ID NO: 67 - DNA, 4645 bp, Artificial Sequence
  Synthetic Polynucleotide
ttggccactccctctctgcgcgctcgctcgctcactgaggccgggcgaccaaaggtcgcccgacgcccgggctttgcccgggcggcctcagtgagcgagcgagcgcgcagagagggagtggccaactccatcactaggggttcctatcgattgaattccaggcgcgccatcctgcaggtattgacgtcaataatgacgtatgttcccatagtaacgccaatagggactttccattgacgtcaatgggtggagtatttacggtaaactgcccacttggcagtacatcaagtgtatcatatgccaagtacgccccctattgacgtcaatgacggtaaatggcccgcctggcattatgcccagtacatgaccttatgggactttcctacttggcagtacatctacgtattagtcatcgctattaccatggtcgaggtgagccccacgttctgcttcactctccccatctcccccccctccccacccccaattttgtatttatttattttttaattattttgtgcagcgatgggggcggggggggggggggggcgcgcgccaggcggggcggggcggggcgaggggcggggcggggcgaggcggagaggtgcggcggcagccaatcagagcggcgcgctccgaaagtttccttttatggcgaggcggcggcggcggcggccctataaaaagcgaagcgcgcggcgggcgggagtcgctgcgcgctgccttcgccccgtgccccgctccgccgccgcctcgcgccgcccgccccggctctgactgaccgcgttactcccacaggtgagcgggcgggacggcccttctcctccgggctgtaattagcgcttggtttaatgacggcttgtttcttttctgtggctgcgtgaaagccttgaggggctccgggagggccctttgtgcggggggagcggctcggggctgtccgcggggggacggctgccttcgggggggacggggcagggcggggttcggcttctggcgtgtgaccggcggctctagagcctctgctaaccatgttcatgccttcttctttttcctacagctcctgggcaacgtgctggttattgtgctgtctcatcattttggcaaagaattgtacaggatatcttgctagcacgccaccatggtttcttactgggacaccggcgtgctgctgtgtgccctgctttcttgtctgctgctgaccggctctagcagcggctctgataccggcagacccttcgtggaaatgtacagcgagatccccgagatcatccacatgaccgagggcagagagctggtcatcccttgcagagtgacaagccccaacatcaccgtgactctgaagaagttccctctggacacactgatccccgacggcaagagaatcatctgggacagccggaagggcttcatcatcagcaacgccacctacaaagagatcggcctgctgacctgtgaagccaccgtgaatggccacctgtacaagaccaactacctgacacacagacagaccaacaccatcatcgacgtggtgctgagccctagccacggcattgaactgtctgtgggcgagaagctggtgctgaactgtaccgccagaaccgagctgaacgtgggcatcgacttcaactgggagtaccccagcagcaagcaccagcacaagaaactggtcaaccgggacctgaaaacccagagcggcagcgagatgaagaaattcctgagcaccctgaccatcgacggcgtgaccagaagtgaccagggcctgtacacatgtgccgccagctctggcctgatgaccaagaaaaacagcaccttcgtgcgggtgcacgagaaggacaagacccacacctgtcctccatgtcctgctccagaactgctcggcggaccttccgtgttcctgtttcctccaaagcctaaggacaccctgatgatcagcagaacccctgaagtgacctgcgtggtggtggatgtgtcccacgaggatcccgaagtgaagttcaattggtacgtggacggcgtggaagtgcacaacgccaagaccaagcctagagaggaacagtacaatagcacctacagagtggtgtccgtgctgaccgtgctgcaccaggattggctgaacggcaaagagtacaagtgcaaggtgtccaacaaggccctgcctgctcctatcgagaaaaccatctccaaggccaagggccagcctagggaaccccaggtttacacactgcctccaagcagggacgagctgacaaagaaccaggtgtccctgacctgcctggtcaagggcttctacccttccgatatcgccgtggaatgggagagcaatggccagcctgagaacaactacaagacaacccctcctgtgctggacagcgacggctcattcttcctgtacagcaagctgacagtggacaagagcagatggcagcagggcaacgtgttcagctgctccgtgatgcacgaggccctgcacaaccactacacccagaagtccctgagcctgtctcctggcaaacggaagagaagaggcagcggcgaaggcagaggatccctgcttacatgtggcgacgtggaagagaaccccggacctatggttctgcagacccaggtgttcatcagcctgctgctgtggatctctggcgcctacggcagctatgtgctgacacagcctccatccgtgtctgtggctccaggacagaccgccagaattacctgcggcggcaacaacatcggcagcaagagcgtgcactggtatcagcagaagcctggacaggctccagtgctggtggtgtacgacgacagcgatagacctagcggcatccccgagagattcagcggcagcaattccggcaataccgccacactgaccatcagcagagtggaagctggcgacgaggccgactactactgccaagtgtgggatagcagcagcgaccactgggttttcggcggaggcaccaaactgacagtgctgagcagcgcctctacaaagggccctagtgtgttccctctggctcccagcagcaagtctacatctggcggaacagccgctctgggctgcctcgtgaaggattactttcccgagcctgtgaccgtgtcctggaatagcggagcactgacaagcggcgtgcacacctttccagctgtgctgcaaagcagcggcctgtactctctgtccagcgtggtcacagtgccaagctctagcctgggcacccagacctacatctgcaatgtgaaccacaagcctagcaacaccaaggtcgacaagaaggtggaacccaagagctgtggcggcagctctggttctggatctggcagcacaggcacatctagctctggcaccggaacaagcgctggcacaactggcacatctgccagcacaagcggatctggaagtggcggaggcggaggatctggtggcggtggatctgcaggcggaactgctacagctggcgcttctagtggaagccaggtgcagctggttcagtctggcgccgaagtgaaaaagcctggcgcctctgtgaaggtgtcctgcaaggccagcggctacacctttaccggctactacatgcactgggtccgacaggcaccaggacagggacttgaatggatgggctggatcaaccccaatagcggcggcaccaattacgcccagaaattccagggcagagtgaccatgaccagagacaccagcatcagcaccgcctacatggaactgagccggctgagatccgatgacaccgccgtgtactactgcgccagatctcccaatccttactactacgacagcagcgggtactactacccaggcgcctttgatatctggggccagggcaccatggtcaccgtgtcatctgcatctgtggccgctcctagcgtgttcatcttcccaccttccgacgaacagctgaagtccggcacagcctctgtcgtgtgcctgctgaacaacttctaccccagagaagccaaagtgcagtggaaggtggacaacgccctgcagagcggcaatagccaagagagcgtgaccgagcaggacagcaaggactctacctacagcctgagcagcaccctgacactgagcaaggccgattacgagaagcacaaggtgtacgcctgcgaagtgacacaccagggcctgtctagccctgtgaccaagagcttcaatcggggcgagtgcgacaagacccacacctaagccacgcgtaacacgtgcatgcgagagatctgcggccgcgagctcggggatccagacatgataagatacattgatgagtttggacaaaccacaactagaatgcagtgaaaaaaatgctttatttgtgaaatttgtgatgctattgctttatttgtaaccattataagctgcaataaacaagttaacaacaacaattgcattcattttatgtttcaggttcagggggaggtgtgggaggttttttaaagcaagtaaaacctctacaaatgtggtatggctgattatgatcaatgcatcctagccggaggaacccctagtgatggagttggccactccctctctgcgcgctcgctcgctcactgaggccgcccgggcaaagcccgggcgtcgggcgacctttggtcgcccggcctcagtgagcgagcgagcgcgcagagagggagtggccaa

SEQ ID NO: 68 - DNA, 3834 bp, Artificial Sequence
  Synthetic Polynucleotide
ttggccactccctctctgcgcgctcgctcgctcactgaggccgggcgaccaaaggtcgcccgacgcccgggctttgcccgggcggcctcagtgagcgagcgagcgcgcagagagggagtggccaactccatcactaggggttcctatcgattgaattccccggggatccactagttattaatagtaatcaattacggggtcattagttcatagcccatatatggagttccgcgttacataacttacggtaaatggcccgcctggctgaccgcccaacgacccccgcccattgacgtcaataatgacgtatgttcccatagtaacgccaatagggactttccattgacgtcaatgggtggagtatttacggtaaactgcccacttggcagtacatcaagtgtatcatatgccaagtacgccccctattgacgtcaatgacggtaaatggcccgcctggcattatgcccagtacatgaccttatgggactttcctacttggcagtacatctacgtattagtcatcgctattaccatggtcgaggtgagccccacgttctgcttcactctccccatctcccccccctccccacccccaattttgtatttatttattttttaattattttgtgcagcgatgggggcggggggggggggggggcgcgcgccaggcggggcggggcggggcgaggggcggggcggggcgaggcggagaggtgcggcggcagccaatcagagcggcgcgctccgaaagtttccttttatggcgaggcggcggcggcggcggccctataaaaagcgaagcgcgcggcgggcggggagtcgctgcgacgctgccttcgccccgtgccccgctccgccgccgcctcgcgccgcccgccccggctctgactgaccgcgttactcccacaggtgagcgggcgggacggcccttctcctccgggctgtaattagcgcttggtttaatgacggcttgtttcttttctgtggctgcgtgaaagccttgaggggctccgggagggccctttgtgcggggggagcggctcggggggtgcgtgcgtgtgtgtgtgcgtggggagcgccgcgtgcggctccgcgctgcccggcggctgtgagcgctgcgggcgcggcgcggggctttgtgcgctccgcagtgtgcgcgaggggagcgcggccgggggcggtgccccgcggtgcggggggggctgcgaggggaacaaaggctgcgtgcggggtgtgtgcgtgggggggtgagcagggggtgtgggcgcgtcggtcgggctgcaaccccccctgcacccccctccccgagttgctgagcacggcccggcttcgggtgcggggctccgtacggggcgtggcgcggggctcgccgtgccgggcggggggtggcggcaggtgggggtgccgggcggggcggggccgcctcgggccggggagggctcgggggaggggcgcggcggcccccggagcgccggcgcgacttcttaacccaacagaaggctcgagaaggtatattgctgttgacagtgagcggcttactcattgtatgaacatttagtgaagccacagatgtaaatgttcatacaatgagtaagctgcctactgcctcggacttcaaggggctagaattcgcggctgtcgaggcgcggcgagccgcagccattgccttttatggtaatcgtgcgagagggcgcagggacttcctttgtcccaaatctgtgcggagccgaaatctgggaggcgccgccgcaccccctctagcgggcgcggggcgaagcggtgcggcgccggcaggaaggaaatgggcggggagggccttcgtgcgtcgccgcgccgccgtccccttctccctctccagcctcggggctgtccgcggggggacggctgccttcgggggggacggggcagggcggggttcggcttctggcgtgtgaccggcggctctagagcctctgctaaccatgttcatgccttcttctttttcctacagtctagagtcgacctgcaggtggatatcttggctagcacgccaccatggtttcttactgggacaccggcgtgctgctgtgtgccctgctttcttgtctgctgctgaccggctctagcagcggctctgataccggcagacccttcgtggaaatgtacagcgagatccccgagatcatccacatgaccgagggcagagagctggtcatcccttgcagagtgacaagccccaacatcaccgtgactctgaagaagttccctctggacacactgatccccgacggcaagagaatcatctgggacagccggaagggcttcatcatcagcaacgccacctacaaagagatcggcctgctgacctgtgaagccaccgtgaatggccacctgtacaagaccaactacctgacacacagacagaccaacaccatcatcgacgtggtgctgagccctagccacggcattgaactgtctgtgggcgagaagctggtgctgaactgtaccgccagaaccgagctgaacgtgggcatcgacttcaactgggagtaccccagcagcaagcaccagcacaagaaactggtcaaccgggacctgaaaacccagagcggcagcgagatgaagaaattcctgagcaccctgaccatcgacggcgtgaccagaagtgaccagggcctgtacacatgtgccgccagctctggcctgatgaccaagaaaaacagcaccttcgtgcgggtgcacgagaaggacaagacccacacctgtcctccatgtcctgctccagaactgctcggcggaccttccgtgttcctgtttcctccaaagcctaaggacaccctgatgatcagcagaacccctgaagtgacctgcgtggtggtggatgtgtcccacgaggatcccgaagtgaagttcaattggtacgtggacggcgtggaagtgcacaacgccaagaccaagcctagagaggaacagtacaatagcacctacagagtggtgtccgtgctgaccgtgctgcaccaggattggctgaacggcaaagagtacaagtgcaaggtgtccaacaaggccctgcctgctcctatcgagaaaaccatctccaaggccaagggccagcctagggaaccccaggtttacacactgcctccaagcagggacgagctgacaaagaaccaggtgtccctgacctgcctggtcaagggcttctacccttccgatatcgccgtggaatgggagagcaatggccagcctgagaacaactacaagacaacccctcctgtgctggacagcgacggctcattcttcctgtacagcaagctgacagtggacaagagcagatggcagcagggcaacgtgttcagctgctccgtgatgcacgaggccctgcacaaccactacacccagaagtccctgagcctgtctcctggcaaatgagccacgcgtaacacgtgggggatccagacatgataagatacattgatgagtttggacaaaccacaactagaatgcagtgaaaaaaatgctttatttgtgaaatttgtgatgctattgctttatttgtaaccattataagctgcaataaacaagttaacaacaacaattgcattcattttatgtttcaggttcagggggaggtgtgggaggttttttaaagcaagtaaaacctctacaaatgtggtatggctgattatgatcaatgcatggccggccggaggaacccctagtgatggagttggccactccctctctgcgcgctcgctcgctcactgaggccgcccgggcaaagcccgggcgtcgggcgacctttggtcgcccggcctcagtgagcgagcgagcgcgcagagagggagtggccaa

SEQ ID NO: 69 - DNA, 3834 bp, Artificial Sequence
  Synthetic Polynucleotide
ttggccactccctctctgcgcgctcgctcgctcactgaggccgggcgaccaaaggtcgcccgacgcccgggctttgcccgggcggcctcagtgagcgagcgagcgcgcagagagggagtggccaactccatcactaggggttcctatcgattgaattccccggggatccactagttattaatagtaatcaattacggggtcattagttcatagcccatatatggagttccgcgttacataacttacggtaaatggcccgcctggctgaccgcccaacgacccccgcccattgacgtcaataatgacgtatgttcccatagtaacgccaatagggactttccattgacgtcaatgggtggagtatttacggtaaactgcccacttggcagtacatcaagtgtatcatatgccaagtacgccccctattgacgtcaatgacggtaaatggcccgcctggcattatgcccagtacatgaccttatgggactttcctacttggcagtacatctacgtattagtcatcgctattaccatggtcgaggtgagccccacgttctgcttcactctccccatctcccccccctccccacccccaattttgtatttatttattttttaattattttgtgcagcgatgggggcggggggggggggggggcgcgcgccaggcggggcggggcggggcgaggggcggggcggggcgaggcggagaggtgcggcggcagccaatcagagcggcgcgctccgaaagtttccttttatggcgaggcggcggcggcggcggccctataaaaagcgaagcgcgcggcgggcggggagtcgctgcgacgctgccttcgccccgtgccccgctccgccgccgcctcgcgccgcccgccccggctctgactgaccgcgttactcccacaggtgagcgggcgggacggcccttctcctccgggctgtaattagcgcttggtttaatgacggcttgtttcttttctgtggctgcgtgaaagccttgaggggctccgggagggccctttgtgcggggggagcggctcggggggtgcgtgcgtgtgtgtgtgcgtggggagcgccgcgtgcggctccgcgctgcccggcggctgtgagcgctgcgggcgcggcgcggggctttgtgcgctccgcagtgtgcgcgaggggagcgcggccgggggcggtgccccgcggtgcggggggggctgcgaggggaacaaaggctgcgtgcggggtgtgtgcgtgggggggtgagcagggggtgtgggcgcgtcggtcgggctgcaaccccccctgcacccccctccccgagttgctgagcacggcccggcttcgggtgcggggctccgtacggggcgtggcgcggggctcgccgtgccgggcggggggtggcggcaggtgggggtgccgggcggggcggggccgcctcgggccggggagggctcgggggaggggcgcggcggcccccggagcgccggcgcgacttcttaacccaacagaaggctcgagaaggtatattgctgttgacagtgagcggctacctcagcaagacgttatttagtgaagccacagatgtaaataacgtcttgctgaggtagctgcctactgcctcggacttcaaggggctagaattcgcggctgtcgaggcgcggcgagccgcagccattgccttttatggtaatcgtgcgagagggcgcagggacttcctttgtcccaaatctgtgcggagccgaaatctgggaggcgccgccgcaccccctctagcgggcgcggggcgaagcggtgcggcgccggcaggaaggaaatgggcggggagggccttcgtgcgtcgccgcgccgccgtccccttctccctctccagcctcggggctgtccgcggggggacggctgccttcgggggggacggggcagggcggggttcggcttctggcgtgtgaccggcggctctagagcctctgctaaccatgttcatgccttcttctttttcctacagtctagagtcgacctgcaggtggatatcttggctagcacgccaccatggtttcttactgggacaccggcgtgctgctgtgtgccctgctttcttgtctgctgctgaccggctctagcagcggctctgataccggcagacccttcgtggaaatgtacagcgagatccccgagatcatccacatgaccgagggcagagagctggtcatcccttgcagagtgacaagccccaacatcaccgtgactctgaagaagttccctctggacacactgatccccgacggcaagagaatcatctgggacagccggaagggcttcatcatcagcaacgccacctacaaagagatcggcctgctgacctgtgaagccaccgtgaatggccacctgtacaagaccaactacctgacacacagacagaccaacaccatcatcgacgtggtgctgagccctagccacggcattgaactgtctgtgggcgagaagctggtgctgaactgtaccgccagaaccgagctgaacgtgggcatcgacttcaactgggagtaccccagcagcaagcaccagcacaagaaactggtcaaccgggacctgaaaacccagagcggcagcgagatgaagaaattcctgagcaccctgaccatcgacggcgtgaccagaagtgaccagggcctgtacacatgtgccgccagctctggcctgatgaccaagaaaaacagcaccttcgtgcgggtgcacgagaaggacaagacccacacctgtcctccatgtcctgctccagaactgctcggcggaccttccgtgttcctgtttcctccaaagcctaaggacaccctgatgatcagcagaacccctgaagtgacctgcgtggtggtggatgtgtcccacgaggatcccgaagtgaagttcaattggtacgtggacggcgtggaagtgcacaacgccaagaccaagcctagagaggaacagtacaatagcacctacagagtggtgtccgtgctgaccgtgctgcaccaggattggctgaacggcaaagagtacaagtgcaaggtgtccaacaaggccctgcctgctcctatcgagaaaaccatctccaaggccaagggccagcctagggaaccccaggtttacacactgcctccaagcagggacgagctgacaaagaaccaggtgtccctgacctgcctggtcaagggcttctacccttccgatatcgccgtggaatgggagagcaatggccagcctgagaacaactacaagacaacccctcctgtgctggacagcgacggctcattcttcctgtacagcaagctgacagtggacaagagcagatggcagcagggcaacgtgttcagctgctccgtgatgcacgaggccctgcacaaccactacacccagaagtccctgagcctgtctcctggcaaatgagccacgcgtaacacgtgggggatccagacatgataagatacattgatgagtttggacaaaccacaactagaatgcagtgaaaaaaatgctttatttgtgaaatttgtgatgctattgctttatttgtaaccattataagctgcaataaacaagttaacaacaacaattgcattcattttatgtttcaggttcagggggaggtgtgggaggttttttaaagcaagtaaaacctctacaaatgtggtatggctgattatgatcaatgcatggccggccggaggaacccctagtgatggagttggccactccctctctgcgcgctcgctcgctcactgaggccgcccgggcaaagcccgggcgtcgggcgacctttggtcgcccggcctcagtgagcgagcgagcgcgcagagagggagtggccaa

SEQ ID NO: 70 - DNA, 3834 bp, Artificial Sequence
  Synthetic Polynucleotide
ttggccactccctctctgcgcgctcgctcgctcactgaggccgggcgaccaaaggtcgcccgacgcccgggctttgcccgggcggcctcagtgagcgagcgagcgcgcagagagggagtggccaactccatcactaggggttcctatcgattgaattccccggggatccactagttattaatagtaatcaattacggggtcattagttcatagcccatatatggagttccgcgttacataacttacggtaaatggcccgcctggctgaccgcccaacgacccccgcccattgacgtcaataatgacgtatgttcccatagtaacgccaatagggactttccattgacgtcaatgggtggagtatttacggtaaactgcccacttggcagtacatcaagtgtatcatatgccaagtacgccccctattgacgtcaatgacggtaaatggcccgcctggcattatgcccagtacatgaccttatgggactttcctacttggcagtacatctacgtattagtcatcgctattaccatggtcgaggtgagccccacgttctgcttcactctccccatctcccccccctccccacccccaattttgtatttatttattttttaattattttgtgcagcgatgggggcggggggggggggggggcgcgcgccaggcggggcggggcggggcgaggggcggggcggggcgaggcggagaggtgcggcggcagccaatcagagcggcgcgctccgaaagtttccttttatggcgaggcggcggcggcggcggccctataaaaagcgaagcgcgcggcgggcggggagtcgctgcgacgctgccttcgccccgtgccccgctccgccgccgcctcgcgccgcccgccccggctctgactgaccgcgttactcccacaggtgagcgggcgggacggcccttctcctccgggctgtaattagcgcttggtttaatgacggcttgtttcttttctgtggctgcgtgaaagccttgaggggctccgggagggccctttgtgcggggggagcggctcggggggtgcgtgcgtgtgtgtgtgcgtggggagcgccgcgtgcggctccgcgctgcccggcggctgtgagcgctgcgggcgcggcgcggggctttgtgcgctccgcagtgtgcgcgaggggagcgcggccgggggcggtgccccgcggtgcggggggggctgcgaggggaacaaaggctgcgtgcggggtgtgtgcgtgggggggtgagcagggggtgtgggcgcgtcggtcgggctgcaaccccccctgcacccccctccccgagttgctgagcacggcccggcttcgggtgcggggctccgtacggggcgtggcgcggggctcgccgtgccgggcggggggtggcggcaggtgggggtgccgggcggggcggggccgcctcgggccggggagggctcgggggaggggcgcggcggcccccggagcgccggcgcgacttcttaacccaacagaaggctcgagaaggtatattgctgttgacagtgagcgcaccgtgtgggctgagtttaactagtgaagccacagatgtagttaaactcagcccacacggtgtgcctactgcctcggacttcaaggggctagaattcgcggctgtcgaggcgcggcgagccgcagccattgccttttatggtaatcgtgcgagagggcgcagggacttcctttgtcccaaatctgtgcggagccgaaatctgggaggcgccgccgcaccccctctagcgggcgcggggcgaagcggtgcggcgccggcaggaaggaaatgggcggggagggccttcgtgcgtcgccgcgccgccgtccccttctccctctccagcctcggggctgtccgcggggggacggctgccttcgggggggacggggcagggcggggttcggcttctggcgtgtgaccggcggctctagagcctctgctaaccatgttcatgccttcttctttttcctacagtctagagtcgacctgcaggtggatatcttggctagcacgccaccatggtttcttactgggacaccggcgtgctgctgtgtgccctgctttcttgtctgctgctgaccggctctagcagcggctctgataccggcagacccttcgtggaaatgtacagcgagatccccgagatcatccacatgaccgagggcagagagctggtcatcccttgcagagtgacaagccccaacatcaccgtgactctgaagaagttccctctggacacactgatccccgacggcaagagaatcatctgggacagccggaagggcttcatcatcagcaacgccacctacaaagagatcggcctgctgacctgtgaagccaccgtgaatggccacctgtacaagaccaactacctgacacacagacagaccaacaccatcatcgacgtggtgctgagccctagccacggcattgaactgtctgtgggcgagaagctggtgctgaactgtaccgccagaaccgagctgaacgtgggcatcgacttcaactgggagtaccccagcagcaagcaccagcacaagaaactggtcaaccgggacctgaaaacccagagcggcagcgagatgaagaaattcctgagcaccctgaccatcgacggcgtgaccagaagtgaccagggcctgtacacatgtgccgccagctctggcctgatgaccaagaaaaacagcaccttcgtgcgggtgcacgagaaggacaagacccacacctgtcctccatgtcctgctccagaactgctcggcggaccttccgtgttcctgtttcctccaaagcctaaggacaccctgatgatcagcagaacccctgaagtgacctgcgtggtggtggatgtgtcccacgaggatcccgaagtgaagttcaattggtacgtggacggcgtggaagtgcacaacgccaagaccaagcctagagaggaacagtacaatagcacctacagagtggtgtccgtgctgaccgtgctgcaccaggattggctgaacggcaaagagtacaagtgcaaggtgtccaacaaggccctgcctgctcctatcgagaaaaccatctccaaggccaagggccagcctagggaaccccaggtttacacactgcctccaagcagggacgagctgacaaagaaccaggtgtccctgacctgcctggtcaagggcttctacccttccgatatcgccgtggaatgggagagcaatggccagcctgagaacaactacaagacaacccctcctgtgctggacagcgacggctcattcttcctgtacagcaagctgacagtggacaagagcagatggcagcagggcaacgtgttcagctgctccgtgatgcacgaggccctgcacaaccactacacccagaagtccctgagcctgtctcctggcaaatgagccacgcgtaacacgtgggggatccagacatgataagatacattgatgagtttggacaaaccacaactagaatgcagtgaaaaaaatgctttatttgtgaaatttgtgatgctattgctttatttgtaaccattataagctgcaataaacaagttaacaacaacaattgcattcattttatgtttcaggttcagggggaggtgtgggaggttttttaaagcaagtaaaacctctacaaatgtggtatggctgattatgatcaatgcatggccggccggaggaacccctagtgatggagttggccactccctctctgcgcgctcgctcgctcactgaggccgcccgggcaaagcccgggcgtcgggcgacctttggtcgcccggcctcagtgagcgagcgagcgcgcagagagggagtggccaa

SEQ ID NO: 71 - protein, 8 aa, Artificial Sequence
  Synthetic Polypeptide
DYKDDDDK

SEQ ID NO: 72 - RNA, 22 nt, Artificial Sequence
  Reverse Transcriptase PCR primer
aauguucauacaaugaguaagc

SEQ ID NO: 73 - RNA, 22 nt, Artificial Sequence
  Reverse Transcriptase PCR Primer
aauaacgucuugcugagguagc

SEQ ID NO: 74 - protein, 7 aa, Artificial Sequence
  Synthetic Polypeptide
ISDQTKH

SEQ ID NO: 75 - protein, 10 aa, Artificial Sequence
  Synthetic Polypeptide
  misc_feature (1)..(2): Xaa is a A, L, G, S, T, P, or absent
  misc_feature (10)..(10): Xaa is a A, L, G, S, T, P, or absent
XXISDQTKHX